European Patent Specification EP 3 481 433 B1, published July 3, 2024. Title: AAV2-MEDIATED GENE DELIVERY OF SFASL AS A NEUROPROTECTIVE THERAPY IN GLAUCOMA. Applicant: University of Massachusetts Massachusetts Eye and Ear Infirmary. Application Not Yet Assigned. The sequence listing filed with the application follows.

SEQUENCE LISTING (29 sequences)

SEQ ID NO: 1 - protein, 735 aa, adeno-associated virus 2 [sequence omitted]

SEQ ID NO: 2 - DNA, 465 bp, Homo Sapiens
gagaagcaaataggccaccccagtccaccccctgaaaaaaaggagctgaggaaagtggcccatttaacaggcaagtccaactcaaggtccatgcctctggaatgggaagacacctatggaattgtcctgctttctggagtgaagtataagaagggtggccttgtgatcaatgaaactgggctgtactttgtatattccaaagtatacttccggggtcaatcttgcaacaacctgcccctgagccacaaggtctacatgaggaactctaagtatccccaggatctggtgatgatggaggggaagatgatgagctactgcactactgggcagatgtgggcccgcagcagctacctgggggcagtgttcaatcttaccagtgctgatcatttatatgtcaacgtatctgagctctctctggtcaattttgaggaatctcagacgtttttcggcttatataagctctaa

SEQ ID NO: 3 - protein, 154 aa, Homo Sapiens
EKQIGHPSPPPEKKELRKVAHLTGKSNSRSMPLEWEDTYGIVLLSGVKYKKGGLVINETGLYFVYSKVYFRGQSCNNLPLSHKVYMRNSKYPQDLVMMEGKMMSYCTTGQMWARSSYLGAVFNLTSADHLYVNVSELSLVNFEESQTFFGLYKL

SEQ ID NO: 4 - DNA, 359 bp, Simian virus 40
tctcccccccctccccacccccaattttgtatttatttattttttaattattttgtgcagcgatgggggcggggggggggggggggggggcgcgcgccaggcggggcggggcggggcgaggggcggggcggggcgaggcggagaggtgcggcggcagccaatcagagcggcgcgctccgaaagtttccttttatggcgaggcggcggcggcggcggccctataaaaagcgaagcgcgcggcgggcgggagcgggatcagccaccgcggtggcggccctagagtcgatcgaggaactgaaaaaccagaaagttaactggtaagtttagtctttttgtcttttatttcaggtcccggatcc

SEQ ID NO: 5 - DNA, 9276 bp, Artificial Sequence
  Synthetic Polynucleotide
ctgcgcgctcgctcgctcactgaggccgcccgggcaaagcccgggcgtcgggcgacctttggtcgcccggcctcagtgagcgagcgagcgcgcagagagggacgcgcgagcgagcgagtgactccggcgggcccgtttcgggcccgcagcccgctggaaaccagcgggccggagtcactcgctcgctcgcgcgtctctccgagtgtagccatgctctaggaagatcaattcggtacaattcacgcgtcgacattgattattgactctggtcgttacataacttacggtaaatggcccgccctcacatcggtacgagatccttctagttaagccatgttaagtgcgcagctgtaactaataactgagaccagcaatgtattgaatgccatttaccgggcggtggctgaccgcccaacgaccccgcccattgacgtcaataatgacgtatgttcccatagtaacgccaatagggactttccattgacgtcaatgggtggagtaccgactggcgggttgctggggcgggtaactgcagttattactgcatacaagggtatcattgcggttatccctgaaaggtaactgcagttacccacctatttacggtaaactgcccacttggcagtacatcaagtgtatcatatgccaagtacgccccctattgacgtcaatgacggtaaatggcccgcctggcattataaatgccatttgacgggtgaaccgtcatgtagttcacatagtatacggttcatgcgggggataactgcagttactgccatttaccgggcggaccgtaattgcccagtacatgaccttatgggactttcctacttggcagtacatctactcgaggccacgttctgcttcactctccccatctcccccccctccccaccccacgggtcatgtactggaataccctgaaaggatgaaccgtcatgtagatgagctccggtgcaagacgaagtgagaggggtagaggggggggaggggtggggcaattttgtatttatttattttttaattattttgtgcagcgatgggggcggggggggggggggggggggcgcgcgccaggcggggcggggcggggcgagggttaaaacataaataaataaaaaattaataaaacacgtcgctacccccgccccccccccccccccccccgcgcgcggtccgccccgccccgccccgctccggcggggcggggcgaggcggagaggtgcggcggcagccaatcagagcggcgcgctccgaaagtttccttttatggcgaggcggcggcggcggcggccctaccgccccgccccgctccgcctctccacgccgccgtcggttagtctcgccgcgcgaggctttcaaaggaaaataccgctccgccgccgccgccgccgggattaaaaagcgaagcgcgcggcgggcgggagcgggatcagccaccgcggtggcggccctagagtcgatcgaggaactgaaaaaccagaaagttaactggtaaatttttcgcttcgcgcgccgcccgccctcgccctagtcggtggcgccaccgccgggatctcagctagctccttgactttttggtctttcaattgaccattgtttagtctttttgtcttttatttcaggtccccggatccatggctcaactttctgcccagaggcgcatgaagctaatggccctgcagctgctgctgtggccaaatcagaaaaacagaaaataaagtccaggggcctaggtaccgagttgaaagacgggtctccgcgtacttcgattaccgggacgtcgacgacgacaccgaaagtgcactatggtcaggacgagaggccgttcccctggtcactgtcagcgctctggaattcgaaaagcaaatagccaaccccagtacaccctctgaaaatttcacgtgataccagtcctgctctccggcaaggggaccagtgacagtcgcgagaccttaagcttttcgtttatcggttggggtcatgtgggagacttttaaaagagccgaggagtgtggcccatttaacagggaacccccactcaaggtccatccctctggaatgggaagacacatatggaaccgctctgatctctggattttctcggctcctcacaccgggtaaattgtcccttgggggtgagttccaggtagggagaccttacccttctgtgtataccttggcgagactagagacctgtgaagtataagaaaggtggccttgtgatcaacgaaactgggttgtacttcgtgtattccaaagtatacttccggggtcagtcctgcaacaaccagcccccacttcatattctttccaccggaacactagttgctttgacccaacatgaagcacataaggtttcatatgaaggccccagtcaggacgttgttggtcggggtaaaccacaaggtctatatgaggaactctaagtatcctgaggatctggtgctaatggaggagaagaggttgaactactgcactactggacagatatgggcatttggtgttccagatatactccttgagattcataggactcctagaccacgattacctcctcttctccaacttgatgacgtgatgacctgtctatacccgccacagcagctacctgggggcagtattcaatcttaccagtgctgaccatttatatgtcaacatatctcaactctctctgatcaattttgaggaatctaagggtgtcgtcgatggacccccgtcataagttagaatggtcacgactggtaaatatacagttgtatagagttgagagagactagttaaaactccttagattcacctttttcggcttatataagcttatcgataccgtcgactagagctcgctgatcagcctcgactgtgccttctagttgccagccatctgttgtttgcccctggaaaaagccgaatatattcgaatagctatggcagctgatctcgagcgactagtcggagctgacacggaagatcaacggtcggtagacaacaaacggggtcccccgtgccttccttgaccctggaaggtgccactcccactgtcctttcctaataaaatgaggaaattgcatcgcattgtctgagtaggtgtcattctaagggggcacggaaggaactgggaccttccacggtgagggtgacaggaaaggattattttactcctttaacgtagcgtaacagactcatccacagtaagatttctggggggtggggtggggcaggacagcaagggggaggattgggaagacaattaggtagataagtagcatggcgggttaatcattaactacaaggaaccaagaccccccaccccaccccgtcctgtcgttccccctcctaacccttctgttaatccatctattcatcgtaccgcccaattagtaattgatgttccttggcctagtgatggagttggccactccctctctgcgcgctcgctcgctcactgaggccgggcgaccaaaggtcgcccgacgcccgggctttgcccgggcggccggatcactacctcaaccggtgagggagagacgcgcgagcgagcgagtgactccggcccgctggtttccagcgggctgcgggcccgaaacgggcccgccggtcagtgagcgagcgagcgcgcagccttaattaacctaattcactggccgtcgttttacaacgtcgtgactgggaaaaccctggcgttacccaacttaatcagtcactcgctcgctcgcgcgtcggaattaattggattaagtgaccggcagcaaaatgttgcagcactgacccttttgggaccgcaatgggttgaattaggccttgcagcacatccccctttcgccagctggcgtaatagcgaagaggcccgcaccgatcgcccttcccaacagttgcgcagcctgaatggcgaatgggacggaacgtcgtgtagggggaaagcggtcgaccgcattatcgcttctccgggcgtggctagcgggaagggttgtcaacgcgtcggacttaccgcttaccctcgcgccctgtagcggcgcattaagcgcggcgggtgtggtggttacgcgcagcgtgaccgctacacttgccagcgccctagcgcccgctcctttcgctttcgcgcgggacatcgccgcgtaattcgcgccgcccacaccaccaatgcgcgtcgcactggcgatgtgaacggtcgcgggatcgcgggcgaggaaagcgaaagttcccttcctttctcgccacgttcgccggctttccccgtcaagctctaaatcgggggctccctttagggttccgatttagtgctttacggcacctcgaccaagggaaggaaagagcggtgcaagcggccgaaaggggcagttcgagatttagcccccgagggaaatcccaaggctaaatcacgaaatgccgtggagctggccaaaaaacttgattagggtgatggttcacgtagtgggccatcgccctgatagacggtttttcgccctttgacgttggagtccacgttctttaatagtggggttttttgaactaatcccactaccaagtgcatcacccggtagcgggactatctgccaaaaagcgggaaactgcaacctcaggtgcaagaaattatcaccactcttgttccaaactggaacaacactcaaccctatctcggtctattcttttgatttataagggattttgccgatttcggcctattggttaaaaaatgagtgagaacaaggtttgaccttgttgtgagttgggatagagccagataagaaaactaaatattccctaaaacggctaaagccggataaccaattttttactcctgatttaacaaaaatttaacgcgaattttaacaaaatattaacgcttacaatttaggtggcacttttcggggaaatgtgcgcggaacccctatttgtttgactaaattgtttttaaattgcgcttaaaattgttttataattgcgaatgttaaatccaccgtgaaaagcccctttacacgcgccttggggataaacaaaatttttctaaatacattcaaatatgtatccgctcatgagacaataaccctgataaatgcttcaataatattgaaaaaggaagagtatgagtattcaacattaaaaagatttatgtaagtttatacataggcgagtactctgttattgggactatttacgaagttattataactttttccttctcatactcataagttgtattccgtgtcgcccttattcccttttttgcggcattttgccttcctgtttttgctcacccagaaacgctggtgaaagtaaaagatgctgaagatcagttggaaggcacagcgggaataagggaaaaaacgccgtaaaacggaaggacaaaaacgagtgggtctttgcgaccactttcattttctacgacttctagtcaaccgtgcacgagtgggttacatcgaactggatctcaacagcggtaagatccttgagagttttcgccccgaagaacgttttccaatgatgagcacttttaaagtcacgtgctcacccaatgtagcttgacctagagttgtcgccattctaggaactctcaaaagcggggcttcttgcaaaaggttactactcgtgaaaatttcatctgctatgtggcgcggtattatcccgtattgacgccgggcaagagcaactcggtcgccgcatacactattctcagaatgacttggttgagtactcaccaagacgatacaccgcgccataatagggcataactgcggcccgttctcgttgagccagcggcgtatgtgataagagtcttactgaaccaactcatgagtggtgtcacagaaaagcatcttacggatggcatgacagtaagagaattatgcagtgctgccataaccatgagtgataacactgcggccaacttacttctgacaacagtgtcttttcgtagaatgcctaccgtactgtcattctcttaatacgtcacgacggtattggtactcactattgtgacgccggttgaatgaagactgttcgatcggaggaccgaaggagctaaccgcttttttgcacaacatgggggatcatgtaactcgccttgatcgttgggaaccggagctgaatgaagccataccgctagcctcctggcttcctcgattggcgaaaaaacgtgttgtaccccctagtacattgagcggaactagcaacccttggcctcgacttacttcggtatggaaacgacgagcgtgacaccacgatgcctgtagcaatggcaacaacgttgcgcaaactattaactggcgaactacttactctagcttcccggcaacaattatttgctgctcgcactgtggtgctacggacatcgttaccgttgttgcaacgcgtttgataattgaccgcttgatgaatgagatcgaagggccgttgttaatatagactggatggaggcggataaagttgcaggaccacttctgcgctcggcccttccggctggctggtttattgctgataaatctggagccggtgagcgtgtatctgacctacctccgcctatttcaacgtcctggtgaagacgcgagccgggaaggccgaccgaccaaataacgactatttagacctcggccactcgcacggtctcgcggtatcattgcagcactggggccagatggtaagccctcccgtatcgtagttatctacacgacggggagtcaggcaactatggatgaacgaaaccagagcgccatagtaacgtcgtgaccccggtctaccattcgggagggcatagcatcaatagatgtgctgcccctcagtccgttgatacctacttgcttttagacagatcgctgagataggtgcctcactgattaagcattggtaactgtcagaccaagtttactcatatatactttagattgatttaaaacttcattttatctgtctagcgactctatccacggagtgactaattcgtaaccattgacagtctggttcaaatgagtatatatgaaatctaactaaattttgaagtaaaataatttaaaaggatctaggtgaagatcctttttgataatctcatgaccaaaatcccttaacgtgagttttcgttccactgagcgtcagaccccgtagaaaattaaattttcctagatccacttctaggaaaaactattagagtactggttttagggaattgcactcaaaagcaaggtgactcgcagtctggggcatctttagatcaaaggatcttcttgagatcctttttttctgcgcgtaatctgctgcttgcaaacaaaaaaaccaccgctaccagcggtggtttgtttgccggatcatctagtttcctagaagaactctaggaaaaaaagacgcgcattagacgacgaacgtttgtttttttggtggcgatggtcgccaccaaacaaacggcctagtagagctaccaactctttttccgaaggtaactggcttcagcagagcgcagataccaaatactgttcttctagtgtagccgtagttaggccaccacttcaagtctcgatggttgagaaaaaggcttccattgaccgaagtcgtctcgcgtctatggtttatgacaagaagatcacatcggcatcaatccggtggtgaagttcaactctgtagcaccgcctacatacctcgctctgctaatcctgttaccagtggctgctgccagtggcgataagtcgtgtcttaccgggttggactcaagacttgagacatcgtggcggatgtatggagcgagacgattaggacaatggtcaccgacgacggtcaccgctattcagcacagaatggcccaacctgagttctggatagttaccggataaggcgcagcggtcgggctgaacggggggttcgtgcacacagcccagcttggagcgaacgacctacaccgaactgagatacctacactatcaatggcctattccgcgtcgccagcccgacttgccccccaagcacgtgtgtcgggtcgaacctcgcttgctggatgtggcttgactctatggatgtgcgtgagctatgagaaagcgccacgcttcccgaagggagaaaggcggacaggtatccggtaagcggcagggtcggaacaggagagcgcacgagggagcttcgcactcgatactctttcgcggtgcgaagggcttccctctttccgcctgtccataggccattcgccgtcccagccttgtcctctcgcgtgctccctcgaaccagggggaaacgcctggtatctttatagtcctgtcgggtttcgccacctctgacttgagcgtcgatttttgtgatgctcgtcaggggggcggagcctatggtccccctttgcggaccatagaaatatcaggacagcccaaagcggtggagactgaactcgcagctaaaaacactacgagcagtccccccgcctcggataggaaaaacgccagcaacgcggcctttttacggttcctggccttttgctggccttttgctcacatgttctttcctgcgttatcccctgattctgtggataacctttttgcggtcgttgcgccggaaaaatgccaaggaccggaaaacgaccggaaaacgagtgtacaagaaaggacgcaataggggactaagacacctattccgtattaccgcctttgagtgagctgataccgctcgccgcagccgaacgaccgagcgcagcgagtcagtgagcgaggaagcggaagagcgcccaatacgcggcataatggcggaaactcactcgactatggcgagcggcgtcggcttgctggctcgcgtcgctcagtcactcgctccttcgccttctcgcgggttatgcgaaaccgcctctccccgcgcgttggccgattcattaatgcagctggcacgacaggtttcccgactggaaagcgggcagtgagcgcaacgcaattaatgtgatttggcggagaggggcgcgcaaccggctaagtaattacgtcgaccgtgctgtccaaagggctgacctttcgcccgtcactcgcgttgcgttaattacacttcattaggcaccccaggctttacactttatgcttccggctcgtatgttgtgtggaattgtgagcggataacaatttcacacaggaaacagcaatcgagtgagtaatccgtggggtccgaaatgtgaaatacgaaggccgagcatacaacacaccttaacactcgcctattgttaaagtgtgtcctttgtcctatgaccatgattacgccagatttaattaaggccttaattagggatactggtactaatgcggtctaaattaattccggaattaatcc

SEQ ID NO: 6 - protein, 281 aa, Homo Sapiens
MQQPFNYPYPQIYWVDSSASSPWAPPGTVLPCPTSVPRRPGQRRPPPPPPPPPLPPPPPPPPLPPLPLPPLKKRGNHSTGLCLLVMFFMVLVALVGLGLGMFQLFHLQKELAELRESTSQMHTASSLEKQIGHPSPPPEKKELRKVAHLTGKSNSRSMPLEWEDTYGIVLLSGVKYKKGGLVINETGLYFVYSKVYFRGQSCNNLPLSHKVYMRNSKYPQDLVMMEGKMMSYCTTGQMWARSSYLGAVFNLTSADHLYVNVSELSLVNFEESQTFFGLYKL

SEQ ID NO: 7 - DNA, 846 bp, Homo Sapiens
atgcagcagcccttcaattacccatatccccagatctactgggtggacagcagtgccagctctccctgggcccctccaggcacagttcttccctgtccaacctctgtgcccagaaggcctggtcaaaggaggccaccaccaccaccgccaccgccaccactaccacctccgccgccgccgccaccactgcctccactaccgctgccacccctgaagaagagagggaaccacagcacaggcctgtgtctccttgtgatgtttttcatggttctggttgccttggtaggattgggcctggggatgtttcagctcttccacctacagaaggagctggcagaactccgagagtctaccagccagatgcacacagcatcatctttggagaagcaaataggccaccccagtccaccccctgaaaaaaaggagctgaggaaagtggcccatttaacaggcaagtccaactcaaggtccatgcctctggaatgggaagacacctatggaattgtcctgctttctggagtgaagtataagaagggtggccttgtgatcaatgaaactgggctgtactttgtatattccaaagtatacttccggggtcaatcttgcaacaacctgcccctgagccacaaggtctacatgaggaactctaagtatccccaggatctggtgatgatggaggggaagatgatgagctactgcactactgggcagatgtgggcccgcagcagctacctgggggcagtgttcaatcttaccagtgctgatcatttatatgtcaacgtatctgagctctctctggtcaattttgaggaatctcagacgtttttcggcttatataagctctaa

SEQ ID NO: 8 - DNA, 20 bp, Artificial Sequence
  Synthetic Polynucleotide
gggacagtgacctggactgt

SEQ ID NO: 9 - DNA, 20 bp, Artificial Sequence
  Synthetic Polynucleotide
ctccctttgcagaactcagg

SEQ ID NO: 10 - DNA, 20 bp, Artificial Sequence
  Synthetic Polynucleotide
tgttaccaactgggacgaca

SEQ ID NO: 11 - DNA, 20 bp, Artificial Sequence
  Synthetic Polynucleotide
cttttcacggttggccttag

SEQ ID NO: 12 - DNA, 19 bp, Artificial Sequence
  Synthetic Polynucleotide
ttctgatatagggtcctgc

SEQ ID NO: 13 - DNA, 20 bp, Artificial Sequence
  Synthetic Polynucleotide
tcaccagatccaagaaactc

SEQ ID NO: 14 - DNA, 20 bp, Artificial Sequence
  Synthetic Polynucleotide
caagctgagtgtaactgaag

SEQ ID NO: 15 - DNA, 20 bp, Artificial Sequence
  Synthetic Polynucleotide
ttaaaaggcatcagcaagag

SEQ ID NO: 16 - DNA, 20 bp, Artificial Sequence
  Synthetic Polynucleotide
ggcgctcaatgctggcttca

SEQ ID NO: 17 - DNA, 20 bp, Artificial Sequence
  Synthetic Polynucleotide
tctgcctccagcctcaggtt

SEQ ID NO: 18 - DNA, 24 bp, Artificial Sequence
  Synthetic Polynucleotide
agggtttcatccaggatcgagcag

SEQ ID NO: 19 - DNA, 21 bp, Artificial Sequence
  Synthetic Polynucleotide
atcttccagatggtgagcgag

SEQ ID NO: 20 - DNA, 24 bp, Artificial Sequence
  Synthetic Polynucleotide
ttgtggccttctttgagttcggtg

SEQ ID NO: 21 - DNA, 24 bp, Artificial Sequence
  Synthetic Polynucleotide
ggtgccggttcaggtactcagtca

SEQ ID NO: 22 - DNA, 20 bp, Artificial Sequence
  Synthetic Polynucleotide
gaagttcccggtttcctctc

SEQ ID NO: 23 - DNA, 20 bp, Artificial Sequence
  Synthetic Polynucleotide
gagggcaggatctctcagtg

SEQ ID NO: 24 - DNA, 20 bp, Artificial Sequence
  Synthetic Polynucleotide
tgtcagccaagttcaagctg

SEQ ID NO: 25 - DNA, 22 bp, Artificial Sequence
  Synthetic Polynucleotide
atcttccgaactttctccaggg

SEQ ID NO: 26 - DNA, 20 bp, Artificial Sequence
  Synthetic Polynucleotide
tgggtagacagcagtgccac

SEQ ID NO: 27 - DNA, 19 bp, Artificial Sequence
  Synthetic Polynucleotide
gcccacaagatggacaggg

SEQ ID NO: 28 - DNA, 22 bp, Artificial Sequence
  Synthetic Polynucleotide
gtcctgcctctggtgcttgctg

SEQ ID NO: 29 - DNA, 17 bp, Artificial Sequence
  Synthetic Polynucleotide
caggttggcatggttga